European Patent Specification EP 3 576 753 B1, published April 17, 2024. Title: STERILE FORMULATION COMPRISING A STABLE PHOSPHOROTHIOATE OLIGONUCLEOTIDE. Applicant: GENE SIGNAL INTERNATIONAL SA VIAUD Éric. The sequence listing filed with the application follows.

SEQUENCE LISTING (28 sequences)

SEQ ID NO: 1 - DNA, 150 bp, Artificial Sequence
  IRS-1 antisense
tagtactcgaggcgcgccgggcccccagcctcgctggccgcgcgcagtacgaagaagcgtttgtgcatgctcttgggtttgcgcaggtagcccaccttgcgcacgtccgagaagccatcgctctccggagggctcgccatgctgccaccg

SEQ ID NO: 2 - DNA, 25 bp, Artificial Sequence
  IRS-1 antisense
tctccggagggctcgccatgctgct

SEQ ID NO: 3 - DNA, 25 bp, Artificial Sequence
  IRS-1 antisense
tatccggagggctcgccatgctgct

SEQ ID NO: 4 - DNA, 24 bp, Artificial Sequence
  IRS-1 antisense
tctccggagggctcgccatgctgc

SEQ ID NO: 5 - DNA, 23 bp, Artificial Sequence
  IRS-1 antisense
tctccggagggctcgccatgctg

SEQ ID NO: 6 - DNA, 22 bp, Artificial Sequence
  IRS-1 antisense
tctccggagggctcgccatgct

SEQ ID NO: 7 - DNA, 21 bp, Artificial Sequence
  IRS-1 antisense
tctccggagggctcgccatgc

SEQ ID NO: 8 - DNA, 20 bp, Artificial Sequence
  IRS-1 antisense
tctccggagggctcgccatg

SEQ ID NO: 9 - DNA, 19 bp, Artificial Sequence
  IRS-1 antisense
tctccggagggctcgccat

SEQ ID NO: 10 - DNA, 24 bp, Artificial Sequence
  IRS-1 antisense
ctccggagggctcgccatgctgct

SEQ ID NO: 11 - DNA, 23 bp, Artificial Sequence
  IRS-1 antisense
tccggagggctcgccatgctgct

SEQ ID NO: 12 - DNA, 22 bp, Artificial Sequence
  IRS-1 antisense
ccggagggctcgccatgctgct

SEQ ID NO: 13 - DNA, 21 bp, Artificial Sequence
  IRS-1 antisense
cggagggctcgccatgctgct

SEQ ID NO: 14 - DNA, 20 bp, Artificial Sequence
  IRS-1 antisense
ggagggctcgccatgctgct

SEQ ID NO: 15 - DNA, 19 bp, Artificial Sequence
  IRS-1 antisense
gagggctcgccatgctgct

SEQ ID NO: 16 - DNA, 18 bp, Artificial Sequence
  IRS-1 antisense
agggctcgccatgctgct

SEQ ID NO: 17 - DNA, 16 bp, Artificial Sequence
  IRS-1 antisense
ggctcgccatgctgct

SEQ ID NO: 18 - DNA, 15 bp, Artificial Sequence
  IRS-1 antisense
gctcgccatgctgct

SEQ ID NO: 19 - DNA, 14 bp, Artificial Sequence
  IRS-1 antisense
ctcgccatgctgct

SEQ ID NO: 20 - DNA, 13 bp, Artificial Sequence
  IRS-1 antisense
tcgccatgctgct

SEQ ID NO: 21 - DNA, 12 bp, Artificial Sequence
  IRS-1 antisense
cgccatgctgct

SEQ ID NO: 22 - DNA, 24 bp, Artificial Sequence
  IRS-1 antisense
tatccggagggctcgccatgctgc

SEQ ID NO: 23 - DNA, 23 bp, Artificial Sequence
  IRS-1 antisense
tatccggagggctcgccatgctg

SEQ ID NO: 24 - DNA, 22 bp, Artificial Sequence
  IRS-1 antisense
tatccggagggctcgccatgct

SEQ ID NO: 25 - DNA, 21 bp, Artificial Sequence
  IRS-1 antisense
tatccggagggctcgccatgc

SEQ ID NO: 26 - DNA, 20 bp, Artificial Sequence
  IRS-1 antisense
tatccggagggctcgccatg

SEQ ID NO: 27 - DNA, 19 bp, Artificial Sequence
  IRS-1 antisense
tatccggagggctcgccat

SEQ ID NO: 28 - DNA, 24 bp, Artificial Sequence
  IRS-1 antisense
atccggagggctcgccatgctgct